European Patent Application EP 4 592 278 A1, published July 30, 2025. Title: Triphenylazole compound. Applicant: Shiratori Pharmaceutical Co., Ltd. The sequence listing filed with the application follows.

SEQUENCE LISTING (4 sequences)

SEQ ID NO: 1 - DNA, 402 bp, Mus musculus
  source 1..402: mol_type = genomic DNA
atggcggacgccttcctgggcacctggaagctagtggacagcaagaatttcgatgactacatgaagtcactcggtgtgggttttgctaccaggcaggtggccagcatgaccaagcctaccacaatcatcgaaaagaatggggacattctcaccctaaaaacacacagcaccttcaagaacacagagatcagctttaagttgggggtggagttcgatgagacaacagcagatgacaggaaggtcaagtccattgtgacactggatggagggaaacttgttcacctgcagaaatgggacgggcaagagaccacacttgtgcgggagctaattgatggaaaactcatcctgacactcacccacggcactgcagtttgcactcgcacttatgagaaagaggcttaa

SEQ ID NO: 2 - DNA, 397 bp, Mus musculus
  source 1..397: mol_type = genomic DNA
atgtgtgatgcttttgtaggtacctggaaacttgtctccagtgaaaactttgatgattatatgaaagaagtaggagtgggctttgccaccaggaaagtggctggcatggccaaacctaacatgatcatcagtgtgaatggggatgtgatcaccattaaatctgaaagtacctttaaaaatactgagatttccttcatactgggccaggaatttgacgaagtcactgcagatgacaggaaagtcaagagcaccataaccttagatgggggtgtcctggtacatgtgcagaaatgggatggaaaatcaaccaccataaagagaaaacgagaggatgataaactggtggtggaatgcgtcatgaaaggcgtcacttccacgagagtttatgagagagcat

SEQ ID NO: 3 - DNA, 408 bp, Mus musculus
  source 1..408: mol_type = genomic DNA
atggccacagttcagcagctggaaggaagatggcgcctggtggacagcaaaggctttgatgaatacatgaaggagctaggagtgggaatagctttgcgaaaaatgggcgcaatggccaagccagattgtatcatcacttgtgatggtaaaaacctcaccataaaaactgagagcactttgaaaacaacacagttttcttgtaccctgggagagaagtttgaagaaaccacagctgatggcagaaaaactcagactgtctgcaactttacagatggtgcattggttcagcatcaggagtgggatgggaaggaaagcacaataacaagaaaattgaaagatgggaaattagtggtggagtgtgtcatgaacaatgtcacctgtactcggatctatgaaaaagtagaataa

SEQ ID NO: 4 - DNA, 399 bp, Mus musculus
  source 1..399: mol_type = genomic DNA
atggtggaggctttctgtgctacctggaagctgaccaacagtcagaactttgatgagtacatgaaggctctaggcgtgggctttgccactaggcaggtgggaaatgtgaccaaaccaacggtaattatcagtcaagaaggagacaaagtggtcatcaggactctcagcacattcaagaacacggagattagtttccagctgggagaagagtttgatgaaaccactgcagatgatagaaactgtaagtctgttgttagcctggatggagacaaacttgttcacatacagaaatgggatggcaaagaaacaaattttgtaagagaaattagggatggcaaaatggttatgacccttacttttggtgatgtggttgctgttcgccactatgagaaggcttaa